European Patent Application EP 4 238 577 A2, published September 6, 2023. Title: COMPOSITIONS FOR ADMINISTRATION OF DIFFERENT DOSES OF RNA. Applicant: BioNTech SE. Application EP 22203154.4, filed October 21, 2022. The sequence listing filed with the application follows.

SEQUENCE LISTING (33 sequences)

SEQ ID NO: 1 - protein, 26 aa, synthetic construct
MRVMAPRTLILLLSGALALTETWAGS

SEQ ID NO: 2 - protein, 55 aa, synthetic construct
IVGIVAGLAVLAVVVIGAVVATVMCRRKSSGGKGGSYSQAASSDSAQGSDVSLTA

SEQ ID NO: 3 - protein, 65 aa, synthetic construct
KKQYIKANSKFIGITELKKLGGGKRGGGKKMTNSVDDALINSTKIYSYFPSVISKVNQGAQGKKL

SEQ ID NO: 4 - protein, 10 aa, synthetic construct
GGSGGGGSGG

SEQ ID NO: 5 - protein, 14 aa, synthetic construct
GSSGGGGSPGGGSS

SEQ ID NO: 6 - RNA, 47 nt, synthetic construct
  source 1..47: mol_type = other RNA
aactagtattcttctggtccccacagactcagagagaacccgccacc

SEQ ID NO: 7 - RNA, 278 nt, synthetic construct
  source 1..278: mol_type = other RNA
ctggtactgcatgcacgcaatgctagctgcccctttcccgtcctgggtaccccgagtctcccccgacctcgggtcccaggtatgctcccacctccacctgccccactcaccacctctgctagttccagacacctcccaagcacgcagcaatgcagctcaaaacgcttagcctagccacacccccacgggaaacagcagtgattaacctttagcaataaacgaaagtttaactaagctatactaaccccagggttggtcaatttcgtgccagccacacc

SEQ ID NO: 8 - RNA, 110 nt, synthetic construct
  source 1..110: mol_type = other RNA
aaaaaaaaaaaaaaaaaaaaaaaaaaaaaagcatatgactaaaaaaaaaaaaaaaaaaaaaaaaaaaaaaaaaaaaaaaaaaaaaaaaaaaaaaaaaaaaaaaaaaaaaa

SEQ ID NO: 9 - protein, 15 aa, synthetic construct
QYIKANSKFIGITEL

SEQ ID NO: 10 - protein, 32 aa, synthetic construct
MTNSVDDALINSTKIYSYFPSVISKVNQGAQG

SEQ ID NO: 11 - protein, 1273 aa, synthetic construct
MFVFLVLLPLVSSQCVNLTTRTQLPPAYTNSFTRGVYYPDKVFRSSVLHSTQDLFLPFFSNVTWFHAIHVSGTNGTKRFDNPVLPFNDGVYFASTEKSNIIRGWIFGTTLDSKTQSLLIVNNATNVVIKVCEFQFCNDPFLGVYYHKNNKSWMESEFRVYSSANNCTFEYVSQPFLMDLEGKQGNFKNLREFVFKNIDGYFKIYSKHTPINLVRDLPQGFSALEPLVDLPIGINITRFQTLLALHRSYLTPGDSSSGWTAGAAAYYVGYLQPRTFLLKYNENGTITDAVDCALDPLSETKCTLKSFTVEKGIYQTSNFRVQPTESIVRFPNITNLCPFGEVFNATRFASVYAWNRKRISNCVADYSVLYNSASFSTFKCYGVSPTKLNDLCFTNVYADSFVIRGDEVRQIAPGQTGKIADYNYKLPDDFTGCVIAWNSNNLDSKVGGNYNYLYRLFRKSNLKPFERDISTEIYQAGSTPCNGVEGFNCYFPLQSYGFQPTNGVGYQPYRVVVLSFELLHAPATVCGPKKSTNLVKNKCVNFNFNGLTGTGVLTESNKKFLPFQQFGRDIADTTDAVRDPQTLEILDITPCSFGGVSVITPGTNTSNQVAVLYQDVNCTEVPVAIHADQLTPTWRVYSTGSNVFQTRAGCLIGAEHVNNSYECDIPIGAGICASYQTQTNSPRRARSVASQSIIAYTMSLGAENSVAYSNNSIAIPTNFTISVTTEILPVSMTKTSVDCTMYICGDSTECSNLLLQYGSFCTQLNRALTGIAVEQDKNTQEVFAQVKQIYKTPPIKDFGGFNFSQILPDPSKPSKRSFIEDLLFNKVTLADAGFIKQYGDCLGDIAARDLICAQKFNGLTVLPPLLTDEMIAQYTSALLAGTITSGWTFGAGAALQIPFAMQMAYRFNGIGVTQNVLYENQKLIANQFNSAIGKIQDSLSSTASALGKLQDVVNQNAQALNTLVKQLSSNFGAISSVLNDILSRLDKVEAEVQIDRLITGRLQSLQTYVTQQLIRAAEIRASANLAATKMSECVLGQSKRVDFCGKGYHLMSFPQSAPHGVVFLHVTYVPAQEKNFTTAPAICHDGKAHFPREGVFVSNGTHWFVTQRNFYEPQIITTDNTFVSGNCDVVIGIVNNTVYDPLQPELDSFKEELDKYFKNHTSPDVDLGDISGINASVVNIQKEIDRLNEVAKNLNESLIDLQELGKYEQYIKWPWYIWLGFIAGLIAIVMVTIMLCCMTSCCSCLKGCCSCGSCCKFDEDDSEPVLKGVKLHYT

SEQ ID NO: 12 - protein, 1273 aa, synthetic construct
MFVFLVLLPLVSSQCVNLTTRTQLPPAYTNSFTRGVYYPDKVFRSSVLHSTQDLFLPFFSNVTWFHAIHVSGTNGTKRFDNPVLPFNDGVYFASTEKSNIIRGWIFGTTLDSKTQSLLIVNNATNVVIKVCEFQFCNDPFLGVYYHKNNKSWMESEFRVYSSANNCTFEYVSQPFLMDLEGKQGNFKNLREFVFKNIDGYFKIYSKHTPINLVRDLPQGFSALEPLVDLPIGINITRFQTLLALHRSYLTPGDSSSGWTAGAAAYYVGYLQPRTFLLKYNENGTITDAVDCALDPLSETKCTLKSFTVEKGIYQTSNFRVQPTESIVRFPNITNLCPFGEVFNATRFASVYAWNRKRISNCVADYSVLYNSASFSTFKCYGVSPTKLNDLCFTNVYADSFVIRGDEVRQIAPGQTGKIADYNYKLPDDFTGCVIAWNSNNLDSKVGGNYNYLYRLFRKSNLKPFERDISTEIYQAGSTPCNGVEGFNCYFPLQSYGFQPTNGVGYQPYRVVVLSFELLHAPATVCGPKKSTNLVKNKCVNFNFNGLTGTGVLTESNKKFLPFQQFGRDIADTTDAVRDPQTLEILDITPCSFGGVSVITPGTNTSNQVAVLYQDVNCTEVPVAIHADQLTPTWRVYSTGSNVFQTRAGCLIGAEHVNNSYECDIPIGAGICASYQTQTNSPRRARSVASQSIIAYTMSLGAENSVAYSNNSIAIPTNFTISVTTEILPVSMTKTSVDCTMYICGDSTECSNLLLQYGSFCTQLNRALTGIAVEQDKNTQEVFAQVKQIYKTPPIKDFGGFNFSQILPDPSKPSKRSFIEDLLFNKVTLADAGFIKQYGDCLGDIAARDLICAQKFNGLTVLPPLLTDEMIAQYTSALLAGTITSGWTFGAGAALQIPFAMQMAYRFNGIGVTQNVLYENQKLIANQFNSAIGKIQDSLSSTASALGKLQDVVNQNAQALNTLVKQLSSNFGAISSVLNDILSRLDPPEAEVQIDRLITGRLQSLQTYVTQQLIRAAEIRASANLAATKMSECVLGQSKRVDFCGKGYHLMSFPQSAPHGVVFLHVTYVPAQEKNFTTAPAICHDGKAHFPREGVFVSNGTHWFVTQRNFYEPQIITTDNTFVSGNCDVVIGIVNNTVYDPLQPELDSFKEELDKYFKNHTSPDVDLGDISGINASVVNIQKEIDRLNEVAKNLNESLIDLQELGKYEQYIKWPWYIWLGFIAGLIAIVMVTIMLCCMTSCCSCLKGCCSCGSCCKFDEDDSEPVLKGVKLHYT

SEQ ID NO: 13 - protein, 41 aa, synthetic construct
GSGYIPEAPRDGQAYVRKDGEWVLLSTFLGRSLEVLFQGPG

SEQ ID NO: 14 - protein, 266 aa, synthetic construct
MFVFLVLLPLVSSQCVVRFPNITNLCPFGEVFNATRFASVYAWNRKRISNCVADYSVLYNSASFSTFKCYGVSPTKLNDLCFTNVYADSFVIRGDEVRQIAPGQTGKIADYNYKLPDDFTGCVIAWNSNNLDSKVGGNYNYLYRLFRKSNLKPFERDISTEIYQAGSTPCNGVEGFNCYFPLQSYGFQPTNGVGYQPYRVVVLSFELLHAPATVCGPKGSPGSGSGSGYIPEAPRDGQAYVRKDGEWVLLSTFLGRSLEVLFQGPG

SEQ ID NO: 15 - protein, 311 aa, synthetic construct
MFVFLVLLPLVSSQCVNLTVRFPNITNLCPFGEVFNATRFASVYAWNRKRISNCVADYSVLYNSASFSTFKCYGVSPTKLNDLCFTNVYADSFVIRGDEVRQIAPGQTGKIADYNYKLPDDFTGCVIAWNSNNLDSKVGGNYNYLYRLFRKSNLKPFERDISTEIYQAGSTPCNGVEGFNCYFPLQSYGFQPTNGVGYQPYRVVVLSFELLHAPATVCGPKGSPGSGSGSGYIPEAPRDGQAYVRKDGEWVLLSTFLGSGSGSEQYIKWPWYIWLGFIAGLIAIVMVTIMLCCMTSCCSCLKGCCSCGSCC

SEQ ID NO: 16 - protein, 314 aa, synthetic construct
MDWIWRILFLVGAATGAHSQMQVRFPNITNLCPFGEVFNATRFASVYAWNRKRISNCVADYSVLYNSASFSTFKCYGVSPTKLNDLCFTNVYADSFVIRGDEVRQIAPGQTGKIADYNYKLPDDFTGCVIAWNSNNLDSKVGGNYNYLYRLFRKSNLKPFERDISTEIYQAGSTPCNGVEGFNCYFPLQSYGFQPTNGVGYQPYRVVVLSFELLHAPATVCGPKGSPGSGSGSGYIPEAPRDGQAYVRKDGEWVLLSTFLGSGSGSEQYIKWPWYIWLGFIAGLIAIVMVTIMLCCMTSCCSCLKGCCSCGSCC

SEQ ID NO: 17 - RNA, 4283 nt, synthetic construct
  source 1..4283: mol_type = other RNA
agaataaactagtattcttctggtccccacagactcagagagaacccgccaccatgttcgtgttcctggtgctgctgcctctggtgtccagccagtgtgtgaacctgaccaccagaacacagctgcctccagcctacaccaacagctttaccagaggcgtgtactaccccgacaaggtgttcagatccagcgtgctgcactctacccaggacctgttcctgcctttcttcagcaacgtgacctggttccacgccatccacgtgtccggcaccaatggcaccaagagattcgacaaccccgtgctgcccttcaacgacggggtgtactttgccagcaccgagaagtccaacatcatcagaggctggatcttcggcaccacactggacagcaagacccagagcctgctgatcgtgaacaacgccaccaacgtggtcatcaaagtgtgcgagttccagttctgcaacgaccccttcctgggcgtctactaccacaagaacaacaagagctggatggaaagcgagttccgggtgtacagcagcgccaacaactgcaccttcgagtacgtgtcccagcctttcctgatggacctggaaggcaagcagggcaacttcaagaacctgcgcgagttcgtgtttaagaacatcgacggctacttcaagatctacagcaagcacacccctatcaacctcgtgcgggatctgcctcagggcttctctgctctggaacccctggtggatctgcccatcggcatcaacatcacccggtttcagacactgctggccctgcacagaagctacctgacacctggcgatagcagcagcggatggacagctggtgccgccgcttactatgtgggctacctgcagcctagaaccttcctgctgaagtacaacgagaacggcaccatcaccgacgccgtggattgtgctctggatcctctgagcgagacaaagtgcaccctgaagtccttcaccgtggaaaagggcatctaccagaccagcaacttccgggtgcagcccaccgaatccatcgtgcggttccccaatatcaccaatctgtgccccttcggcgaggtgttcaatgccaccagattcgcctctgtgtacgcctggaaccggaagcggatcagcaattgcgtggccgactactccgtgctgtacaactccgccagcttcagcaccttcaagtgctacggcgtgtcccctaccaagctgaacgacctgtgcttcacaaacgtgtacgccgacagcttcgtgatccggggagatgaagtgcggcagattgcccctggacagacaggcaagatcgccgactacaactacaagctgcccgacgacttcaccggctgtgtgattgcctggaacagcaacaacctggactccaaagtcggcggcaactacaattacctgtaccggctgttccggaagtccaatctgaagcccttcgagcgggacatctccaccgagatctatcaggccggcagcaccccttgtaacggcgtggaaggcttcaactgctacttcccactgcagtcctacggctttcagcccacaaatggcgtgggctatcagccctacagagtggtggtgctgagcttcgaactgctgcatgcccctgccacagtgtgcggccctaagaaaagcaccaatctcgtgaagaacaaatgcgtgaacttcaacttcaacggcctgaccggcaccggcgtgctgacagagagcaacaagaagttcctgccattccagcagtttggccgggatatcgccgataccacagacgccgttagagatccccagacactggaaatcctggacatcaccccttgcagcttcggcggagtgtctgtgatcacccctggcaccaacaccagcaatcaggtggcagtgctgtaccaggacgtgaactgtaccgaagtgcccgtggccattcacgccgatcagctgacacctacatggcgggtgtactccaccggcagcaatgtgtttcagaccagagccggctgtctgatcggagccgagcacgtgaacaatagctacgagtgcgacatccccatcggcgctggaatctgcgccagctaccagacacagacaaacagccctcggagagccagaagcgtggccagccagagcatcattgcctacacaatgtctctgggcgccgagaacagcgtggcctactccaacaactctatcgctatccccaccaacttcaccatcagcgtgaccacagagatcctgcctgtgtccatgaccaagaccagcgtggactgcaccatgtacatctgcggcgattccaccgagtgctccaacctgctgctgcagtacggcagcttctgcacccagctgaatagagccctgacagggatcgccgtggaacaggacaagaacacccaagaggtgttcgcccaagtgaagcagatctacaagacccctcctatcaaggacttcggcggcttcaatttcagccagattctgcccgatcctagcaagcccagcaagcggagcttcatcgaggacctgctgttcaacaaagtgacactggccgacgccggcttcatcaagcagtatggcgattgtctgggcgacattgccgccagggatctgatttgcgcccagaagtttaacggactgacagtgctgcctcctctgctgaccgatgagatgatcgcccagtacacatctgccctgctggccggcacaatcacaagcggctggacatttggagcaggcgccgctctgcagatcccctttgctatgcagatggcctaccggttcaacggcatcggagtgacccagaatgtgctgtacgagaaccagaagctgatcgccaaccagttcaacagcgccatcggcaagatccaggacagcctgagcagcacagcaagcgccctgggaaagctgcaggacgtggtcaaccagaatgcccaggcactgaacaccctggtcaagcagctgtcctccaacttcggcgccatcagctctgtgctgaacgatatcctgagcagactggaccctcctgaggccgaggtgcagatcgacagactgatcacaggcagactgcagagcctccagacatacgtgacccagcagctgatcagagccgccgagattagagcctctgccaatctggccgccaccaagatgtctgagtgtgtgctgggccagagcaagagagtggacttttgcggcaagggctaccacctgatgagcttccctcagtctgcccctcacggcgtggtgtttctgcacgtgacatatgtgcccgctcaagagaagaatttcaccaccgctccagccatctgccacgacggcaaagcccactttcctagagaaggcgtgttcgtgtccaacggcacccattggttcgtgacacagcggaacttctacgagccccagatcatcaccaccgacaacaccttcgtgtctggcaactgcgacgtcgtgatcggcattgtgaacaataccgtgtacgaccctctgcagcccgagctggacagcttcaaagaggaactggacaagtactttaagaaccacacaagccccgacgtggacctgggcgatatcagcggaatcaatgccagcgtcgtgaacatccagaaagagatcgaccggctgaacgaggtggccaagaatctgaacgagagcctgatcgacctgcaagaactggggaagtacgagcagtacatcaagtggccctggtacatctggctgggctttatcgccggactgattgccatcgtgatggtcacaatcatgctgtgttgcatgaccagctgctgtagctgcctgaagggctgttgtagctgtggcagctgctgcaagttcgacgaggacgattctgagcccgtgctgaagggcgtgaaactgcactacacatgatgactcgagctggtactgcatgcacgcaatgctagctgcccctttcccgtcctgggtaccccgagtctcccccgacctcgggtcccaggtatgctcccacctccacctgccccactcaccacctctgctagttccagacacctcccaagcacgcagcaatgcagctcaaaacgcttagcctagccacacccccacgggaaacagcagtgattaacctttagcaataaacgaaagtttaactaagctatactaaccccagggttggtcaatttcgtgccagccacaccctggagctagcaaaaaaaaaaaaaaaaaaaaaaaaaaaaaagcatatgactaaaaaaaaaaaaaaaaaaaaaaaaaaaaaaaaaaaaaaaaaaaaaaaaaaaaaaaaaaaaaaaaaaaaaa

SEQ ID NO: 18 - RNA, 1262 nt, synthetic construct
  source 1..1262: mol_type = other RNA
agaataaactagtattcttctggtccccacagactcagagagaacccgccaccatgtttgtgtttcttgtgctgctgcctcttgtgtcttctcagtgtgtggtgagatttccaaatattacaaatctgtgtccatttggagaagtgtttaatgcaacaagatttgcatctgtgtatgcatggaatagaaaaagaatttctaattgtgtggctgattattctgtgctgtataatagtgcttctttttccacatttaaatgttatggagtgtctccaacaaaattaaatgatttatgttttacaaatgtgtatgctgattcttttgtgatcagaggtgatgaagtgagacagattgcccccggacagacaggaaaaattgctgattacaattacaaactgcctgatgattttacaggatgtgtgattgcttggaattctaataatttagattctaaagtgggaggaaattacaattatctgtacagactgtttagaaaatcaaatctgaaaccttttgaaagagatatttcaacagaaatttatcaggctggatcaacaccttgtaatggagtggaaggatttaattgttattttccattacagagctatggatttcagccaaccaatggtgtgggatatcagccatatagagtggtggtgctgtcttttgaactgctgcatgcacctgcaacagtgtgtggacctaaaggctcccccggctccggctccggatctggttatattcctgaagctccaagagatgggcaagcttacgttcgtaaagatggcgaatgggtattactttctacctttttaggccggtccctggaggtgctgttccagggccccggctgatgactcgagctggtactgcatgcacgcaatgctagctgcccctttcccgtcctgggtaccccgagtctcccccgacctcgggtcccaggtatgctcccacctccacctgccccactcaccacctctgctagttccagacacctcccaagcacgcagcaatgcagctcaaaacgcttagcctagccacacccccacgggaaacagcagtgattaacctttagcaataaacgaaagtttaactaagctatactaaccccagggttggtcaatttcgtgccagccacaccctggagctagcaaaaaaaaaaaaaaaaaaaaaaaaaaaaaagcatatgactaaaaaaaaaaaaaaaaaaaaaaaaaaaaaaaaaaaaaaaaaaaaaaaaaaaaaaaaaaaaaaaaaaaaaa

SEQ ID NO: 19 - RNA, 1397 nt, synthetic construct
  source 1..1397: mol_type = other RNA
agaataaactagtattcttctggtccccacagactcagagagaacccgccaccatgtttgtgtttcttgtgctgctgcctcttgtgtcttctcagtgtgtgaatttgacagtgagatttccaaatattacaaatctgtgtccatttggagaagtgtttaatgcaacaagatttgcatctgtgtatgcatggaatagaaaaagaatttctaattgtgtggctgattattctgtgctgtataatagtgcttctttttccacatttaaatgttatggagtgtctccaacaaaattaaatgatttatgttttacaaatgtgtatgctgattcttttgtgatcagaggtgatgaagtgagacagattgcccccggacagacaggaaaaattgctgattacaattacaaactgcctgatgattttacaggatgtgtgattgcttggaattctaataatttagattctaaagtgggaggaaattacaattatctgtacagactgtttagaaaatcaaatctgaaaccttttgaaagagatatttcaacagaaatttatcaggctggatcaacaccttgtaatggagtggaaggatttaattgttattttccattacagagctatggatttcagccaaccaatggtgtgggatatcagccatatagagtggtggtgctgtcttttgaactgctgcatgcacctgcaacagtgtgtggacctaaaggctcccccggctccggctccggatctggttatattcctgaagctccaagagatgggcaagcttacgttcgtaaagatggcgaatgggtattactttctacctttttaggaagcggcagcggatctgaacagtacattaaatggccttggtacatttggcttggatttattgcaggattaattgcaattgtgatggtgacaattatgttatgttgtatgacatcatgttgttcttgtttaaaaggatgttgttcttgtggaagctgttgttgatgactcgagctggtactgcatgcacgcaatgctagctgcccctttcccgtcctgggtaccccgagtctcccccgacctcgggtcccaggtatgctcccacctccacctgccccactcaccacctctgctagttccagacacctcccaagcacgcagcaatgcagctcaaaacgcttagcctagccacacccccacgggaaacagcagtgattaacctttagcaataaacgaaagtttaactaagctatactaaccccagggttggtcaatttcgtgccagccacaccctggagctagcaaaaaaaaaaaaaaaaaaaaaaaaaaaaaagcatatgactaaaaaaaaaaaaaaaaaaaaaaaaaaaaaaaaaaaaaaaaaaaaaaaaaaaaaaaaaaaaaaaaaaaaaa

SEQ ID NO: 20 - RNA, 1406 nt, synthetic construct
  source 1..1406: mol_type = other RNA
agaataaactagtattcttctggtccccacagactcagagagaacccgccaccatggattggatttggagaatcctgttcctcgtgggagccgctacaggagcccactcccagatgcaggtgagatttccaaatattacaaatctgtgtccatttggagaagtgtttaatgcaacaagatttgcatctgtgtatgcatggaatagaaaaagaatttctaattgtgtggctgattattctgtgctgtataatagtgcttctttttccacatttaaatgttatggagtgtctccaacaaaattaaatgatttatgttttacaaatgtgtatgctgattcttttgtgatcagaggtgatgaagtgagacagattgcccccggacagacaggaaaaattgctgattacaattacaaactgcctgatgattttacaggatgtgtgattgcttggaattctaataatttagattctaaagtgggaggaaattacaattatctgtacagactgtttagaaaatcaaatctgaaaccttttgaaagagatatttcaacagaaatttatcaggctggatcaacaccttgtaatggagtggaaggatttaattgttattttccattacagagctatggatttcagccaaccaatggtgtgggatatcagccatatagagtggtggtgctgtcttttgaactgctgcatgcacctgcaacagtgtgtggacctaaaggctcccccggctccggctccggatctggttatattcctgaagctccaagagatgggcaagcttacgttcgtaaagatggcgaatgggtattactttctacctttttaggaagcggcagcggatctgaacagtacattaaatggccttggtacatttggcttggatttattgcaggattaattgcaattgtgatggtgacaattatgttatgttgtatgacatcatgttgttcttgtttaaaaggatgttgttcttgtggaagctgttgttgatgactcgagctggtactgcatgcacgcaatgctagctgcccctttcccgtcctgggtaccccgagtctcccccgacctcgggtcccaggtatgctcccacctccacctgccccactcaccacctctgctagttccagacacctcccaagcacgcagcaatgcagctcaaaacgcttagcctagccacacccccacgggaaacagcagtgattaacctttagcaataaacgaaagtttaactaagctatactaaccccagggttggtcaatttcgtgccagccacaccctggagctagcaaaaaaaaaaaaaaaaaaaaaaaaaaaaaagcatatgactaaaaaaaaaaaaaaaaaaaaaaaaaaaaaaaaaaaaaaaaaaaaaaaaaaaaaaaaaaaaaaaaaaaaaa

SEQ ID NO: 21 - RNA, 3819 nt, synthetic construct
  source 1..3819: mol_type = other RNA
atgttcgtgttcctggtgctgctgcctctggtgtccagccagtgtgtgaacctgaccaccagaacacagctgcctccagcctacaccaacagctttaccagaggcgtgtactaccccgacaaggtgttcagatccagcgtgctgcactctacccaggacctgttcctgcctttcttcagcaacgtgacctggttccacgccatccacgtgtccggcaccaatggcaccaagagattcgacaaccccgtgctgcccttcaacgacggggtgtactttgccagcaccgagaagtccaacatcatcagaggctggatcttcggcaccacactggacagcaagacccagagcctgctgatcgtgaacaacgccaccaacgtggtcatcaaagtgtgcgagttccagttctgcaacgaccccttcctgggcgtctactaccacaagaacaacaagagctggatggaaagcgagttccgggtgtacagcagcgccaacaactgcaccttcgagtacgtgtcccagcctttcctgatggacctggaaggcaagcagggcaacttcaagaacctgcgcgagttcgtgtttaagaacatcgacggctacttcaagatctacagcaagcacacccctatcaacctcgtgcgggatctgcctcagggcttctctgctctggaacccctggtggatctgcccatcggcatcaacatcacccggtttcagacactgctggccctgcacagaagctacctgacacctggcgatagcagcagcggatggacagctggtgccgccgcttactatgtgggctacctgcagcctagaaccttcctgctgaagtacaacgagaacggcaccatcaccgacgccgtggattgtgctctggatcctctgagcgagacaaagtgcaccctgaagtccttcaccgtggaaaagggcatctaccagaccagcaacttccgggtgcagcccaccgaatccatcgtgcggttccccaatatcaccaatctgtgccccttcggcgaggtgttcaatgccaccagattcgcctctgtgtacgcctggaaccggaagcggatcagcaattgcgtggccgactactccgtgctgtacaactccgccagcttcagcaccttcaagtgctacggcgtgtcccctaccaagctgaacgacctgtgcttcacaaacgtgtacgccgacagcttcgtgatccggggagatgaagtgcggcagattgcccctggacagacaggcaagatcgccgactacaactacaagctgcccgacgacttcaccggctgtgtgattgcctggaacagcaacaacctggactccaaagtcggcggcaactacaattacctgtaccggctgttccggaagtccaatctgaagcccttcgagcgggacatctccaccgagatctatcaggccggcagcaccccttgtaacggcgtggaaggcttcaactgctacttcccactgcagtcctacggctttcagcccacaaatggcgtgggctatcagccctacagagtggtggtgctgagcttcgaactgctgcatgcccctgccacagtgtgcggccctaagaaaagcaccaatctcgtgaagaacaaatgcgtgaacttcaacttcaacggcctgaccggcaccggcgtgctgacagagagcaacaagaagttcctgccattccagcagtttggccgggatatcgccgataccacagacgccgttagagatccccagacactggaaatcctggacatcaccccttgcagcttcggcggagtgtctgtgatcacccctggcaccaacaccagcaatcaggtggcagtgctgtaccaggacgtgaactgtaccgaagtgcccgtggccattcacgccgatcagctgacacctacatggcgggtgtactccaccggcagcaatgtgtttcagaccagagccggctgtctgatcggagccgagcacgtgaacaatagctacgagtgcgacatccccatcggcgctggaatctgcgccagctaccagacacagacaaacagccctcggagagccagaagcgtggccagccagagcatcattgcctacacaatgtctctgggcgccgagaacagcgtggcctactccaacaactctatcgctatccccaccaacttcaccatcagcgtgaccacagagatcctgcctgtgtccatgaccaagaccagcgtggactgcaccatgtacatctgcggcgattccaccgagtgctccaacctgctgctgcagtacggcagcttctgcacccagctgaatagagccctgacagggatcgccgtggaacaggacaagaacacccaagaggtgttcgcccaagtgaagcagatctacaagacccctcctatcaaggacttcggcggcttcaatttcagccagattctgcccgatcctagcaagcccagcaagcggagcttcatcgaggacctgctgttcaacaaagtgacactggccgacgccggcttcatcaagcagtatggcgattgtctgggcgacattgccgccagggatctgatttgcgcccagaagtttaacggactgacagtgctgcctcctctgctgaccgatgagatgatcgcccagtacacatctgccctgctggccggcacaatcacaagcggctggacatttggagcaggcgccgctctgcagatcccctttgctatgcagatggcctaccggttcaacggcatcggagtgacccagaatgtgctgtacgagaaccagaagctgatcgccaaccagttcaacagcgccatcggcaagatccaggacagcctgagcagcacagcaagcgccctgggaaagctgcaggacgtggtcaaccagaatgcccaggcactgaacaccctggtcaagcagctgtcctccaacttcggcgccatcagctctgtgctgaacgatatcctgagcagactggaccctcctgaggccgaggtgcagatcgacagactgatcacaggcagactgcagagcctccagacatacgtgacccagcagctgatcagagccgccgagattagagcctctgccaatctggccgccaccaagatgtctgagtgtgtgctgggccagagcaagagagtggacttttgcggcaagggctaccacctgatgagcttccctcagtctgcccctcacggcgtggtgtttctgcacgtgacatatgtgcccgctcaagagaagaatttcaccaccgctccagccatctgccacgacggcaaagcccactttcctagagaaggcgtgttcgtgtccaacggcacccattggttcgtgacacagcggaacttctacgagccccagatcatcaccaccgacaacaccttcgtgtctggcaactgcgacgtcgtgatcggcattgtgaacaataccgtgtacgaccctctgcagcccgagctggacagcttcaaagaggaactggacaagtactttaagaaccacacaagccccgacgtggacctgggcgatatcagcggaatcaatgccagcgtcgtgaacatccagaaagagatcgaccggctgaacgaggtggccaagaatctgaacgagagcctgatcgacctgcaagaactggggaagtacgagcagtacatcaagtggccctggtacatctggctgggctttatcgccggactgattgccatcgtgatggtcacaatcatgctgtgttgcatgaccagctgctgtagctgcctgaagggctgttgtagctgtggcagctgctgcaagttcgacgaggacgattctgagcccgtgctgaagggcgtgaaactgcactacaca

SEQ ID NO: 22 - protein, 1270 aa, synthetic construct
MFVFLVLLPLVSSQCVNFTTRTQLPPAYTNSFTRGVYYPDKVFRSSVLHSTQDLFLPFFSNVTWFHAIHVSGTNGTKRFANPVLPFNDGVYFASTEKSNIIRGWIFGTTLDSKTQSLLIVNNATNVVIKVCEFQFCNDPFLGVYYHKNNKSWMESEFRVYSSANNCTFEYVSQPFLMDLEGKQGNFKNLREFVFKNIDGYFKIYSKHTPINLVRGLPQGFSALEPLVDLPIGINITRFQTLHISYLTPGDSSSGWTAGAAAYYVGYLQPRTFLLKYNENGTITDAVDCALDPLSETKCTLKSFTVEKGIYQTSNFRVQPTESIVRFPNITNLCPFGEVFNATRFASVYAWNRKRISNCVADYSVLYNSASFSTFKCYGVSPTKLNDLCFTNVYADSFVIRGDEVRQIAPGQTGNIADYNYKLPDDFTGCVIAWNSNNLDSKVGGNYNYLYRLFRKSNLKPFERDISTEIYQAGSTPCNGVKGFNCYFPLQSYGFQPTYGVGYQPYRVVVLSFELLHAPATVCGPKKSTNLVKNKCVNFNFNGLTGTGVLTESNKKFLPFQQFGRDIADTTDAVRDPQTLEILDITPCSFGGVSVITPGTNTSNQVAVLYQGVNCTEVPVAIHADQLTPTWRVYSTGSNVFQTRAGCLIGAEHVNNSYECDIPIGAGICASYQTQTNSPRRARSVASQSIIAYTMSLGVENSVAYSNNSIAIPTNFTISVTTEILPVSMTKTSVDCTMYICGDSTECSNLLLQYGSFCTQLNRALTGIAVEQDKNTQEVFAQVKQIYKTPPIKDFGGFNFSQILPDPSKPSKRSFIEDLLFNKVTLADAGFIKQYGDCLGDIAARDLICAQKFNGLTVLPPLLTDEMIAQYTSALLAGTITSGWTFGAGAALQIPFAMQMAYRFNGIGVTQNVLYENQKLIANQFNSAIGKIQDSLSSTASALGKLQDVVNQNAQALNTLVKQLSSNFGAISSVLNDILSRLDPPEAEVQIDRLITGRLQSLQTYVTQQLIRAAEIRASANLAATKMSECVLGQSKRVDFCGKGYHLMSFPQSAPHGVVFLHVTYVPAQEKNFTTAPAICHDGKAHFPREGVFVSNGTHWFVTQRNFYEPQIITTDNTFVSGNCDVVIGIVNNTVYDPLQPELDSFKEELDKYFKNHTSPDVDLGDISGINASVVNIQKEIDRLNEVAKNLNESLIDLQELGKYEQYIKWPWYIWLGFIAGLIAIVMVTIMLCCMTSCCSCLKGCCSCGSCCKFDEDDSEPVLKGVKLHYT

SEQ ID NO: 23 - RNA, 3817 nt, synthetic construct
  source 1..3817: mol_type = other RNA
atgttcgtgttcctggtgctgctgcctctggtgtccagccagtgtgtgaacttcaccaccagaacacagctgcctccagcctacaccaacagctttaccagaggcgtgtactaccccgacaaggtgttcagatccagcgtgctgcactctacccaggacctgttcctgcctttcttcagcaacgtgacctggttccacgccatccacgtgtccggcaccaatggcaccaagagattcgccaaccccgtgctgcccttcaacgacggggtgtactttgccagcaccgagaagtccaacatcatcagaggctggatcttcggcaccacactggacagcaagacccagagcctgctgatcgtgaacaacgccaccaacgtggtcatcaaagtgtgcgagttccagttctgcaacgaccccttcctgggcgtctactaccacaagaacaacaagagctggatggaaagcgagttccgggtgtacagcagcgccaacaactgcaccttcgagtacgtgtcccagcctttcctgatggacctggaaggcaagcagggcaacttcaagaacctgcgcgagttcgtgtttaagaacatcgacggctacttcaagatctacagcaagcacacccctatcaacctcgtgcggggcctgcctcagggcttctctgctctggaacccctggtggatctgcccatcggcatcaacatcacccggtttcagacactgcacatcagctacctgacacctggcgatagcagcagcggatggacagctggtgccgccgcttactatgtgggctacctgcagcctagaaccttcctgctgaagtacaacgagaacggcaccatcaccgacgccgtggattgtgctctggatcctctgagcgagacaaagtgcaccctgaagtccttcaccgtggaaaagggcatctaccagaccagcaacttccgggtgcagcccaccgaatccatcgtgcggttccccaatatcaccaatctgtgccccttcggcgaggtgttcaatgccaccagattcgcctctgtgtacgcctggaaccggaagcggatcagcaattgcgtggccgactactccgtgctgtacaactccgccagcttcagcaccttcaagtgctacggcgtgtcccctaccaagctgaacgacctgtgcttcacaaacgtgtacgccgacagcttcgtgatccggggagatgaagtgcggcagattgcccctggacagacaggcaacatcgccgactacaactacaagctgcccgacgacttcaccggctgtgtgattgcctggaacagcaacaacctggactccaaagtcggcggcaactacaattacctgtaccggctgttccggaagtccaatctgaagcccttcgagcgggacatctccaccgagatctatcaggccggcagcaccccttgtaacggcgtgaagggcttcaactgctacttcccactgcagtcctacggctttcagcccacatacggcgtgggctatcagccctacagagtggtggtgctgagcttcgaactgctgcatgcccctgccacagtgtgcggccctaagaaaagcaccaatctcgtgaagaacaaatgcgtgaacttcaacttcaacggcctgaccggcaccggcgtgctgacagagagcaacaagaagttcctgccattccagcagtttggccgggatatcgccgataccacagacgccgttagagatccccagacactggaaatcctggacatcaccccttgcagcttcggcggagtgtctgtgatcacccctggcaccaacaccagcaatcaggtggcagtgctgtaccagggcgtgaactgtaccgaagtgcccgtggccattcacgccgatcagctgacacctacatggcgggtgtactccaccggcagcaatgtgtttcagaccagagccggctgtctgatcggagccgagcacgtgaacaatagctacgagtgcgacatccccatcggcgctggaatctgcgccagctaccagacacagacaaacagccctcggagagccagaagcgtggccagccagagcatcattgcctacacaatgtctctgggcgtcgagaacagcgtggcctactccaacaactctatcgctatccccaccaacttcaccatcagcgtgaccacagagatcctgcctgtgtccatgaccaagaccagcgtggactgcaccatgtacatctgcggcgattccaccgagtgctccaacctgctgctgcagtacggcagcttctgcacccagctgaatagagccctgacagggatcgccgtggaacaggacaagaacacccaagaggtgttcgcccaagtgaagcagatctacaagacccctcctatcaaggacttcggcggcttcaatttcagccagattctgcccgatcctagcaagcccagcaagcggagcttcatcgaggacctgctgttcaacaaagtgacactggccgacgccggcttcatcaagcagtatggcgattgtctgggcgacattgccgccagggatctgatttgcgcccagaagtttaacggactgacagtgctgcctcctctgctgaccgatgagatgatcgcccagtacacatctgccctgctggccggcacaatcacaagcggctggacatttggagcaggcgccgctctgcagatcccctttgctatgcagatggcctaccggttcaacggcatcggagtgacccagaatgtgctgtacgagaaccagaagctgatcgccaaccagttcaacagcgccatcggcaagatccaggacagcctgagcagcacagcaagcgccctgggaaagctgcaggacgtggtcaaccagaatgcccaggcactgaacaccctggtcaagcagctgtcctccaacttcggcgccatcagctctgtgctgaacgatatcctgagcagactggaccctcctgaggccgaggtgcagatcgacagactgatcacaggcagactgcagagcctccagacatacgtgacccagcagctgatcagagccgccgagattagagcctctgccaatctggccgccaccaagatgtctgagtgtgtgctgggccagagcaagagagtggacttttgcggcaagggctaccacctgatgagcttccctcagtctgcccctcacggcgtggtgtttctgcacgtgacatatgtgcccgctcaagagaagaatttcaccaccgctccagccatctgccacgacggcaaagcccactttcctagagaaggcgtgttcgtgtccaacggcacccattggttcgtgacacagcggaacttctacgagccccagatcatcaccaccgacaacaccttcgtgtctggcaactgcgacgtcgtgatcggcattgtgaacaataccgtgtacgaccctctgcagcccgagctggacagcttcaaagaggaactggacaagtactttaagaaccacacaagccccgacgtggacctgggcgatatcagcggaatcaatgccagcgtcgtgaacatccagaaagagatcgaccggctgaacgaggtggccaagaatctgaacgagagcctgatcgacctgcaagaactggggaagtacgagcagtacatcaagtggccctggtacatctggctgggctttatcgccggactgattgccatcgtgatggtcacaatcatgctgtgttgcatgaccagctgctgtagctgcctgaagggctgttgtagctgtggcagctgctgcaagttcgacgaggacgattctgagcccgtgctgaagggcgtgaaactgcactacacatgatgac

SEQ ID NO: 24 - RNA, 4274 nt, synthetic construct
  source 1..4274: mol_type = other RNA
agaataaactagtattcttctggtccccacagactcagagagaacccgccaccatgttcgtgttcctggtgctgctgcctctggtgtccagccagtgtgtgaacttcaccaccagaacacagctgcctccagcctacaccaacagctttaccagaggcgtgtactaccccgacaaggtgttcagatccagcgtgctgcactctacccaggacctgttcctgcctttcttcagcaacgtgacctggttccacgccatccacgtgtccggcaccaatggcaccaagagattcgccaaccccgtgctgcccttcaacgacggggtgtactttgccagcaccgagaagtccaacatcatcagaggctggatcttcggcaccacactggacagcaagacccagagcctgctgatcgtgaacaacgccaccaacgtggtcatcaaagtgtgcgagttccagttctgcaacgaccccttcctgggcgtctactaccacaagaacaacaagagctggatggaaagcgagttccgggtgtacagcagcgccaacaactgcaccttcgagtacgtgtcccagcctttcctgatggacctggaaggcaagcagggcaacttcaagaacctgcgcgagttcgtgtttaagaacatcgacggctacttcaagatctacagcaagcacacccctatcaacctcgtgcggggcctgcctcagggcttctctgctctggaacccctggtggatctgcccatcggcatcaacatcacccggtttcagacactgcacatcagctacctgacacctggcgatagcagcagcggatggacagctggtgccgccgcttactatgtgggctacctgcagcctagaaccttcctgctgaagtacaacgagaacggcaccatcaccgacgccgtggattgtgctctggatcctctgagcgagacaaagtgcaccctgaagtccttcaccgtggaaaagggcatctaccagaccagcaacttccgggtgcagcccaccgaatccatcgtgcggttccccaatatcaccaatctgtgccccttcggcgaggtgttcaatgccaccagattcgcctctgtgtacgcctggaaccggaagcggatcagcaattgcgtggccgactactccgtgctgtacaactccgccagcttcagcaccttcaagtgctacggcgtgtcccctaccaagctgaacgacctgtgcttcacaaacgtgtacgccgacagcttcgtgatccggggagatgaagtgcggcagattgcccctggacagacaggcaacatcgccgactacaactacaagctgcccgacgacttcaccggctgtgtgattgcctggaacagcaacaacctggactccaaagtcggcggcaactacaattacctgtaccggctgttccggaagtccaatctgaagcccttcgagcgggacatctccaccgagatctatcaggccggcagcaccccttgtaacggcgtgaagggcttcaactgctacttcccactgcagtcctacggctttcagcccacatacggcgtgggctatcagccctacagagtggtggtgctgagcttcgaactgctgcatgcccctgccacagtgtgcggccctaagaaaagcaccaatctcgtgaagaacaaatgcgtgaacttcaacttcaacggcctgaccggcaccggcgtgctgacagagagcaacaagaagttcctgccattccagcagtttggccgggatatcgccgataccacagacgccgttagagatccccagacactggaaatcctggacatcaccccttgcagcttcggcggagtgtctgtgatcacccctggcaccaacaccagcaatcaggtggcagtgctgtaccagggcgtgaactgtaccgaagtgcccgtggccattcacgccgatcagctgacacctacatggcgggtgtactccaccggcagcaatgtgtttcagaccagagccggctgtctgatcggagccgagcacgtgaacaatagctacgagtgcgacatccccatcggcgctggaatctgcgccagctaccagacacagacaaacagccctcggagagccagaagcgtggccagccagagcatcattgcctacacaatgtctctgggcgtcgagaacagcgtggcctactccaacaactctatcgctatccccaccaacttcaccatcagcgtgaccacagagatcctgcctgtgtccatgaccaagaccagcgtggactgcaccatgtacatctgcggcgattccaccgagtgctccaacctgctgctgcagtacggcagcttctgcacccagctgaatagagccctgacagggatcgccgtggaacaggacaagaacacccaagaggtgttcgcccaagtgaagcagatctacaagacccctcctatcaaggacttcggcggcttcaatttcagccagattctgcccgatcctagcaagcccagcaagcggagcttcatcgaggacctgctgttcaacaaagtgacactggccgacgccggcttcatcaagcagtatggcgattgtctgggcgacattgccgccagggatctgatttgcgcccagaagtttaacggactgacagtgctgcctcctctgctgaccgatgagatgatcgcccagtacacatctgccctgctggccggcacaatcacaagcggctggacatttggagcaggcgccgctctgcagatcccctttgctatgcagatggcctaccggttcaacggcatcggagtgacccagaatgtgctgtacgagaaccagaagctgatcgccaaccagttcaacagcgccatcggcaagatccaggacagcctgagcagcacagcaagcgccctgggaaagctgcaggacgtggtcaaccagaatgcccaggcactgaacaccctggtcaagcagctgtcctccaacttcggcgccatcagctctgtgctgaacgatatcctgagcagactggaccctcctgaggccgaggtgcagatcgacagactgatcacaggcagactgcagagcctccagacatacgtgacccagcagctgatcagagccgccgagattagagcctctgccaatctggccgccaccaagatgtctgagtgtgtgctgggccagagcaagagagtggacttttgcggcaagggctaccacctgatgagcttccctcagtctgcccctcacggcgtggtgtttctgcacgtgacatatgtgcccgctcaagagaagaatttcaccaccgctccagccatctgccacgacggcaaagcccactttcctagagaaggcgtgttcgtgtccaacggcacccattggttcgtgacacagcggaacttctacgagccccagatcatcaccaccgacaacaccttcgtgtctggcaactgcgacgtcgtgatcggcattgtgaacaataccgtgtacgaccctctgcagcccgagctggacagcttcaaagaggaactggacaagtactttaagaaccacacaagccccgacgtggacctgggcgatatcagcggaatcaatgccagcgtcgtgaacatccagaaagagatcgaccggctgaacgaggtggccaagaatctgaacgagagcctgatcgacctgcaagaactggggaagtacgagcagtacatcaagtggccctggtacatctggctgggctttatcgccggactgattgccatcgtgatggtcacaatcatgctgtgttgcatgaccagctgctgtagctgcctgaagggctgttgtagctgtggcagctgctgcaagttcgacgaggacgattctgagcccgtgctgaagggcgtgaaactgcactacacatgatgactcgagctggtactgcatgcacgcaatgctagctgcccctttcccgtcctgggtaccccgagtctcccccgacctcgggtcccaggtatgctcccacctccacctgccccactcaccacctctgctagttccagacacctcccaagcacgcagcaatgcagctcaaaacgcttagcctagccacacccccacgggaaacagcagtgattaacctttagcaataaacgaaagtttaactaagctatactaaccccagggttggtcaatttcgtgccagccacaccctggagctagcaaaaaaaaaaaaaaaaaaaaaaaaaaaaaagcatatgactaaaaaaaaaaaaaaaaaaaaaaaaaaaaaaaaaaaaaaaaaaaaaaaaaaaaaaaaaaaaaaaaaaaaaa

SEQ ID NO: 25 - protein, 1270 aa, synthetic construct
MFVFLVLLPLVSSQCVNLTTRTQLPPAYTNSFTRGVYYPDKVFRSSVLHSTQDLFLPFFSNVTWFHAISGTNGTKRFDNPVLPFNDGVYFASTEKSNIIRGWIFGTTLDSKTQSLLIVNNATNVVIKVCEFQFCNDPFLGVYHKNNKSWMESEFRVYSSANNCTFEYVSQPFLMDLEGKQGNFKNLREFVFKNIDGYFKIYSKHTPINLVRDLPQGFSALEPLVDLPIGINITRFQTLLALHRSYLTPGDSSSGWTAGAAAYYVGYLQPRTFLLKYNENGTITDAVDCALDPLSETKCTLKSFTVEKGIYQTSNFRVQPTESIVRFPNITNLCPFGEVFNATRFASVYAWNRKRISNCVADYSVLYNSASFSTFKCYGVSPTKLNDLCFTNVYADSFVIRGDEVRQIAPGQTGKIADYNYKLPDDFTGCVIAWNSNNLDSKVGGNYNYLYRLFRKSNLKPFERDISTEIYQAGSTPCNGVEGFNCYFPLQSYGFQPTYGVGYQPYRVVVLSFELLHAPATVCGPKKSTNLVKNKCVNFNFNGLTGTGVLTESNKKFLPFQQFGRDIDDTTDAVRDPQTLEILDITPCSFGGVSVITPGTNTSNQVAVLYQGVNCTEVPVAIHADQLTPTWRVYSTGSNVFQTRAGCLIGAEHVNNSYECDIPIGAGICASYQTQTNSHRRARSVASQSIIAYTMSLGAENSVAYSNNSIAIPINFTISVTTEILPVSMTKTSVDCTMYICGDSTECSNLLLQYGSFCTQLNRALTGIAVEQDKNTQEVFAQVKQIYKTPPIKDFGGFNFSQILPDPSKPSKRSFIEDLLFNKVTLADAGFIKQYGDCLGDIAARDLICAQKFNGLTVLPPLLTDEMIAQYTSALLAGTITSGWTFGAGAALQIPFAMQMAYRFNGIGVTQNVLYENQKLIANQFNSAIGKIQDSLSSTASALGKLQDVVNQNAQALNTLVKQLSSNFGAISSVLNDILARLDPPEAEVQIDRLITGRLQSLQTYVTQQLIRAAEIRASANLAATKMSECVLGQSKRVDFCGKGYHLMSFPQSAPHGVVFLHVTYVPAQEKNFTTAPAICHDGKAHFPREGVFVSNGTHWFVTQRNFYEPQIITTHNTFVSGNCDVVIGIVNNTVYDPLQPELDSFKEELDKYFKNHTSPDVDLGDISGINASVVNIQKEIDRLNEVAKNLNESLIDLQELGKYEQYIKWPWYIWLGFIAGLIAIVMVTIMLCCMTSCCSCLKGCCSCGSCCKFDEDDSEPVLKGVKLHYT

SEQ ID NO: 26 - RNA, 3816 nt, synthetic construct
  source 1..3816: mol_type = other RNA
atgttcgtgttcctggtgctgctgcctctggtgtccagccagtgtgtgaacctgaccaccagaacacagctgcctccagcctacaccaacagctttaccagaggcgtgtactaccccgacaaggtgttcagatccagcgtgctgcactctacccaggacctgttcctgcctttcttcagcaacgtgacctggttccacgccatctccggcaccaatggcaccaagagattcgacaaccccgtgctgcccttcaacgacggggtgtactttgccagcaccgagaagtccaacatcatcagaggctggatcttcggcaccacactggacagcaagacccagagcctgctgatcgtgaacaacgccaccaacgtggtcatcaaagtgtgcgagttccagttctgcaacgaccccttcctgggcgtctaccacaagaacaacaagagctggatggaaagcgagttccgggtgtacagcagcgccaacaactgcaccttcgagtacgtgtcccagcctttcctgatggacctggaaggcaagcagggcaacttcaagaacctgcgcgagttcgtgtttaagaacatcgacggctacttcaagatctacagcaagcacacccctatcaacctcgtgcgggatctgcctcagggcttctctgctctggaacccctggtggatctgcccatcggcatcaacatcacccggtttcagacactgctggccctgcacagaagctacctgacacctggcgatagcagcagcggatggacagctggtgccgccgcttactatgtgggctacctgcagcctagaaccttcctgctgaagtacaacgagaacggcaccatcaccgacgccgtggattgtgctctggatcctctgagcgagacaaagtgcaccctgaagtccttcaccgtggaaaagggcatctaccagaccagcaacttccgggtgcagcccaccgaatccatcgtgcggttccccaatatcaccaatctgtgccccttcggcgaggtgttcaatgccaccagattcgcctctgtgtacgcctggaaccggaagcggatcagcaattgcgtggccgactactccgtgctgtacaactccgccagcttcagcaccttcaagtgctacggcgtgtcccctaccaagctgaacgacctgtgcttcacaaacgtgtacgccgacagcttcgtgatccggggagatgaagtgcggcagattgcccctggacagacaggcaagatcgccgactacaactacaagctgcccgacgacttcaccggctgtgtgattgcctggaacagcaacaacctggactccaaagtcggcggcaactacaattacctgtaccggctgttccggaagtccaatctgaagcccttcgagcgggacatctccaccgagatctatcaggccggcagcaccccttgtaacggcgtggaaggcttcaactgctacttcccactgcagtcctacggctttcagcccacatacggcgtgggctatcagccctacagagtggtggtgctgagcttcgaactgctgcatgcccctgccacagtgtgcggccctaagaaaagcaccaatctcgtgaagaacaaatgcgtgaacttcaacttcaacggcctgaccggcaccggcgtgctgacagagagcaacaagaagttcctgccattccagcagtttggccgggatatcgacgataccacagacgccgttagagatccccagacactggaaatcctggacatcaccccttgcagcttcggcggagtgtctgtgatcacccctggcaccaacaccagcaatcaggtggcagtgctgtaccagggcgtgaactgtaccgaagtgcccgtggccattcacgccgatcagctgacacctacatggcgggtgtactccaccggcagcaatgtgtttcagaccagagccggctgtctgatcggagccgagcacgtgaacaatagctacgagtgcgacatccccatcggcgctggaatctgcgccagctaccagacacagacaaacagccaccggagagccagaagcgtggccagccagagcatcattgcctacacaatgtctctgggcgccgagaacagcgtggcctactccaacaactctatcgctatccccatcaacttcaccatcagcgtgaccacagagatcctgcctgtgtccatgaccaagaccagcgtggactgcaccatgtacatctgcggcgattccaccgagtgctccaacctgctgctgcagtacggcagcttctgcacccagctgaatagagccctgacagggatcgccgtggaacaggacaagaacacccaagaggtgttcgcccaagtgaagcagatctacaagacccctcctatcaaggacttcggcggcttcaatttcagccagattctgcccgatcctagcaagcccagcaagcggagcttcatcgaggacctgctgttcaacaaagtgacactggccgacgccggcttcatcaagcagtatggcgattgtctgggcgacattgccgccagggatctgatttgcgcccagaagtttaacggactgacagtgctgcctcctctgctgaccgatgagatgatcgcccagtacacatctgccctgctggccggcacaatcacaagcggctggacatttggagcaggcgccgctctgcagatcccctttgctatgcagatggcctaccggttcaacggcatcggagtgacccagaatgtgctgtacgagaaccagaagctgatcgccaaccagttcaacagcgccatcggcaagatccaggacagcctgagcagcacagcaagcgccctgggaaagctgcaggacgtggtcaaccagaatgcccaggcactgaacaccctggtcaagcagctgtcctccaacttcggcgccatcagctctgtgctgaacgatatcctggccagactggaccctcctgaggccgaggtgcagatcgacagactgatcacaggcagactgcagagcctccagacatacgtgacccagcagctgatcagagccgccgagattagagcctctgccaatctggccgccaccaagatgtctgagtgtgtgctgggccagagcaagagagtggacttttgcggcaagggctaccacctgatgagcttccctcagtctgcccctcacggcgtggtgtttctgcacgtgacatatgtgcccgctcaagagaagaatttcaccaccgctccagccatctgccacgacggcaaagcccactttcctagagaaggcgtgttcgtgtccaacggcacccattggttcgtgacacagcggaacttctacgagccccagatcatcaccacccacaacaccttcgtgtctggcaactgcgacgtcgtgatcggcattgtgaacaataccgtgtacgaccctctgcagcccgagctggacagcttcaaagaggaactggacaagtactttaagaaccacacaagccccgacgtggacctgggcgatatcagcggaatcaatgccagcgtcgtgaacatccagaaagagatcgaccggctgaacgaggtggccaagaatctgaacgagagcctgatcgacctgcaagaactggggaagtacgagcagtacatcaagtggccctggtacatctggctgggctttatcgccggactgattgccatcgtgatggtcacaatcatgctgtgttgcatgaccagctgctgtagctgcctgaagggctgttgtagctgtggcagctgctgcaagttcgacgaggacgattctgagcccgtgctgaagggcgtgaaactgcactacacatgatga

SEQ ID NO: 27 - RNA, 4274 nt, synthetic construct
  source 1..4274: mol_type = other RNA
agaataaactagtattcttctggtccccacagactcagagagaacccgccaccatgttcgtgttcctggtgctgctgcctctggtgtccagccagtgtgtgaacctgaccaccagaacacagctgcctccagcctacaccaacagctttaccagaggcgtgtactaccccgacaaggtgttcagatccagcgtgctgcactctacccaggacctgttcctgcctttcttcagcaacgtgacctggttccacgccatctccggcaccaatggcaccaagagattcgacaaccccgtgctgcccttcaacgacggggtgtactttgccagcaccgagaagtccaacatcatcagaggctggatcttcggcaccacactggacagcaagacccagagcctgctgatcgtgaacaacgccaccaacgtggtcatcaaagtgtgcgagttccagttctgcaacgaccccttcctgggcgtctaccacaagaacaacaagagctggatggaaagcgagttccgggtgtacagcagcgccaacaactgcaccttcgagtacgtgtcccagcctttcctgatggacctggaaggcaagcagggcaacttcaagaacctgcgcgagttcgtgtttaagaacatcgacggctacttcaagatctacagcaagcacacccctatcaacctcgtgcgggatctgcctcagggcttctctgctctggaacccctggtggatctgcccatcggcatcaacatcacccggtttcagacactgctggccctgcacagaagctacctgacacctggcgatagcagcagcggatggacagctggtgccgccgcttactatgtgggctacctgcagcctagaaccttcctgctgaagtacaacgagaacggcaccatcaccgacgccgtggattgtgctctggatcctctgagcgagacaaagtgcaccctgaagtccttcaccgtggaaaagggcatctaccagaccagcaacttccgggtgcagcccaccgaatccatcgtgcggttccccaatatcaccaatctgtgccccttcggcgaggtgttcaatgccaccagattcgcctctgtgtacgcctggaaccggaagcggatcagcaattgcgtggccgactactccgtgctgtacaactccgccagcttcagcaccttcaagtgctacggcgtgtcccctaccaagctgaacgacctgtgcttcacaaacgtgtacgccgacagcttcgtgatccggggagatgaagtgcggcagattgcccctggacagacaggcaagatcgccgactacaactacaagctgcccgacgacttcaccggctgtgtgattgcctggaacagcaacaacctggactccaaagtcggcggcaactacaattacctgtaccggctgttccggaagtccaatctgaagcccttcgagcgggacatctccaccgagatctatcaggccggcagcaccccttgtaacggcgtggaaggcttcaactgctacttcccactgcagtcctacggctttcagcccacatacggcgtgggctatcagccctacagagtggtggtgctgagcttcgaactgctgcatgcccctgccacagtgtgcggccctaagaaaagcaccaatctcgtgaagaacaaatgcgtgaacttcaacttcaacggcctgaccggcaccggcgtgctgacagagagcaacaagaagttcctgccattccagcagtttggccgggatatcgacgataccacagacgccgttagagatccccagacactggaaatcctggacatcaccccttgcagcttcggcggagtgtctgtgatcacccctggcaccaacaccagcaatcaggtggcagtgctgtaccagggcgtgaactgtaccgaagtgcccgtggccattcacgccgatcagctgacacctacatggcgggtgtactccaccggcagcaatgtgtttcagaccagagccggctgtctgatcggagccgagcacgtgaacaatagctacgagtgcgacatccccatcggcgctggaatctgcgccagctaccagacacagacaaacagccaccggagagccagaagcgtggccagccagagcatcattgcctacacaatgtctctgggcgccgagaacagcgtggcctactccaacaactctatcgctatccccatcaacttcaccatcagcgtgaccacagagatcctgcctgtgtccatgaccaagaccagcgtggactgcaccatgtacatctgcggcgattccaccgagtgctccaacctgctgctgcagtacggcagcttctgcacccagctgaatagagccctgacagggatcgccgtggaacaggacaagaacacccaagaggtgttcgcccaagtgaagcagatctacaagacccctcctatcaaggacttcggcggcttcaatttcagccagattctgcccgatcctagcaagcccagcaagcggagcttcatcgaggacctgctgttcaacaaagtgacactggccgacgccggcttcatcaagcagtatggcgattgtctgggcgacattgccgccagggatctgatttgcgcccagaagtttaacggactgacagtgctgcctcctctgctgaccgatgagatgatcgcccagtacacatctgccctgctggccggcacaatcacaagcggctggacatttggagcaggcgccgctctgcagatcccctttgctatgcagatggcctaccggttcaacggcatcggagtgacccagaatgtgctgtacgagaaccagaagctgatcgccaaccagttcaacagcgccatcggcaagatccaggacagcctgagcagcacagcaagcgccctgggaaagctgcaggacgtggtcaaccagaatgcccaggcactgaacaccctggtcaagcagctgtcctccaacttcggcgccatcagctctgtgctgaacgatatcctggccagactggaccctcctgaggccgaggtgcagatcgacagactgatcacaggcagactgcagagcctccagacatacgtgacccagcagctgatcagagccgccgagattagagcctctgccaatctggccgccaccaagatgtctgagtgtgtgctgggccagagcaagagagtggacttttgcggcaagggctaccacctgatgagcttccctcagtctgcccctcacggcgtggtgtttctgcacgtgacatatgtgcccgctcaagagaagaatttcaccaccgctccagccatctgccacgacggcaaagcccactttcctagagaaggcgtgttcgtgtccaacggcacccattggttcgtgacacagcggaacttctacgagccccagatcatcaccacccacaacaccttcgtgtctggcaactgcgacgtcgtgatcggcattgtgaacaataccgtgtacgaccctctgcagcccgagctggacagcttcaaagaggaactggacaagtactttaagaaccacacaagccccgacgtggacctgggcgatatcagcggaatcaatgccagcgtcgtgaacatccagaaagagatcgaccggctgaacgaggtggccaagaatctgaacgagagcctgatcgacctgcaagaactggggaagtacgagcagtacatcaagtggccctggtacatctggctgggctttatcgccggactgattgccatcgtgatggtcacaatcatgctgtgttgcatgaccagctgctgtagctgcctgaagggctgttgtagctgtggcagctgctgcaagttcgacgaggacgattctgagcccgtgctgaagggcgtgaaactgcactacacatgatgagatctgctggtactgcatgcacgcaatgctagctgcccctttcccgtcctgggtaccccgagtctcccccgacctcgggtcccaggtatgctcccacctccacctgccccactcaccacctctgctagttccagacacctcccaagcacgcagcaatgcagctcaaaacgcttagcctagccacacccccacgggaaacagcagtgattaacctttagcaataaacgaaagtttaactaagctatactaaccccagggttggtcaatttcgtgccagccacaccctggagctagcaaaaaaaaaaaaaaaaaaaaaaaaaaaaaagcatatgactaaaaaaaaaaaaaaaaaaaaaaaaaaaaaaaaaaaaaaaaaaaaaaaaaaaaaaaaaaaaaaaaaaaaaa

SEQ ID NO: 28 - protein, 1271 aa, synthetic construct
MFVFLVLLPLVSSQCVNLRTRTQLPPAYTNSFTRGVYYPDKVFRSSVLHSTQDLFLPFFSNVTWFHAIHVSGTNGTKRFDNPVLPFNDGVYFASTEKSNIIRGWIFGTTLDSKTQSLLIVNNATNVVIKVCEFQFCNDPFLDVYYHKNNKSWMESGVYSSANNCTFEYVSQPFLMDLEGKQGNFKNLREFVFKNIDGYFKIYSKHTPINLVRDLPQGFSALEPLVDLPIGINITRFQTLLALHRSYLTPGDSSSGWTAGAAAYYVGYLQPRTFLLKYNENGTITDAVDCALDPLSETKCTLKSFTVEKGIYQTSNFRVQPTESIVRFPNITNLCPFGEVFNATRFASVYAWNRKRISNCVADYSVLYNSASFSTFKCYGVSPTKLNDLCFTNVYADSFVIRGDEVRQIAPGQTGKIADYNYKLPDDFTGCVIAWNSNNLDSKVGGNYNYRYRLFRKSNLKPFERDISTEIYQAGSKPCNGVEGFNCYFPLQSYGFQPTNGVGYQPYRVVVLSFELLHAPATVCGPKKSTNLVKNKCVNFNFNGLTGTGVLTESNKKFLPFQQFGRDIADTTDAVRDPQTLEILDITPCSFGGVSVITPGTNTSNQVAVLYQGVNCTEVPVAIHADQLTPTWRVYSTGSNVFQTRAGCLIGAEHVNNSYECDIPIGAGICASYQTQTNSRRRARSVASQSIIAYTMSLGAENSVAYSNNSIAIPTNFTISVTTEILPVSMTKTSVDCTMYICGDSTECSNLLLQYGSFCTQLNRALTGIAVEQDKNTQEVFAQVKQIYKTPPIKDFGGFNFSQILPDPSKPSKRSFIEDLLFNKVTLADAGFIKQYGDCLGDIAARDLICAQKFNGLTVLPPLLTDEMIAQYTSALLAGTITSGWTFGAGAALQIPFAMQMAYRFNGIGVTQNVLYENQKLIANQFNSAIGKIQDSLSSTASALGKLQNVVNQNAQALNTLVKQLSSNFGAISSVLNDILSRLDPPEAEVQIDRLITGRLQSLQTYVTQQLIRAAEIRASANLAATKMSECVLGQSKRVDFCGKGYHLMSFPQSAPHGVVFLHVTYVPAQEKNFTTAPAICHDGKAHFPREGVFVSNGTHWFVTQRNFYEPQIITTDNTFVSGNCDVVIGIVNNTVYDPLQPELDSFKEELDKYFKNHTSPDVDLGDISGINASVVNIQKEIDRLNEVAKNLNESLIDLQELGKYEQYIKWPWYIWLGFIAGLIAIVMVTIMLCCMTSCCSCLKGCCSCGSCCKFDEDDSEPVLKGVKLHYT

SEQ ID NO: 29 - RNA, 4899 nt, synthetic construct
  source 1..4899: mol_type = other RNA
atgttcgtgttcctggtgctgctgcctctggtgtccagccagtgtgtgaacctgagaaccagaacacagctgcctccagcctacaccaacagctttaccagaggcgtgtactaccccgacaaggtgttcagatccagcgtgctgcactctacccaggacctgttcctgcctttcttcagcaacgtgacctggttccacgccatccacgtgtccggcaccaatggcaccaagagattcgacaaccccgtgctgcccttcaacgacggggtgtactttgccagcaccgagaagtccaacatcatcagaggctggatcttcggcaccacactggacagcaagacccagagcctgctgatcgtgaacaacgccaccaacgtggtcatcaaagtgtgcgagttccagttctgcaacgaccccttcctggacgtctactaccacaagaacaacaagagctggatggaaagcggcgtgtacagcagcgccaacaactgcaccttcgagtacgtgtcccagcctttcctgatggacctggaaggcaagcagggcaacttcaagaacctgcgcgagttcgtgtttaagaacatcgacggctacttcaagatctacagcaagcacacccctatcaacctcgtgcgggatctgcctcagggcttctctgctctggaacccctggtggatctgcccatcggcatcaacatcacccggtttcagacactgctggccctgcacagaagctacctgacacctggcgatagcagcagcggatggacagctggtgccgccgcttactatgtgggctacctgcagcctagaaccttcctgctgaagtacaacgagaacggcaccatcaccgacgccgtggattgtgctctggatcctctgagcgagacaaagtgcaccctgaagtccttcaccgtggaaaagggcatctaccagaccagcaacttccgggtgcagcccaccgaatccatcgtgcggttccccaatatcaccaatctgtgccccttcggcgaggtgttcaatgccaccagattcgcctctgtgtacgcctggaaccggaagcggatcagcaattgcgtgatgttcgtgttcctggtgctgctgcctctggtgtccagccagtgtgtgaacctgagaaccagaacacagctgcctccagcctacaccaacagctttaccagaggcgtgtactaccccgacaaggtgttcagatccagcgtgctgcactctacccaggacctgttcctgcctttcttcagcaacgtgacctggttccacgccatccacgtgtccggcaccaatggcaccaagagattcgacaaccccgtgctgcccttcaacgacggggtgtactttgccagcaccgagaagtccaacatcatcagaggctggatcttcggcaccacactggacagcaagacccagagcctgctgatcgtgaacaacgccaccaacgtggtcatcaaagtgtgcgagttccagttctgcaacgaccccttcctggacgtctactaccacaagaacaacaagagctggatggaaagcggcgtgtacagcagcgccaacaactgcaccttcgagtacgtgtcccagcctttcctgatggacctggaaggcaagcagggcaacttcaagaacctgcgcgagttcgtgtttaagaacatcgacggctacttcaagatctacagcaagcacacccctatcaacctcgtgcgggatctgcctcagggcttctctgctctggaacccctggtggatctgcccatcggcatcaacatcacccggtttcagacactgctggccctgcacagaagctacctgacacctggcgatagcagcagcggatggacagctggtgccgccgcttactatgtgggctacctgcagcctagaaccttcctgctgaagtacaacgagaacggcaccatcaccgacgccgtggattgtgctctggatcctctgagcgagacaaagtgcaccctgaagtccttcaccgtggaaaagggcatctaccagaccagcaacttccgggtgcagcccaccgaatccatcgtgcggttccccaatatcaccaatctgtgccccttcggcgaggtgttcaatgccaccagattcgcctctgtgtacgcctggaaccggaagcggatcagcaattgcgtggccgactactccgtgctgtacaactccgccagcttcagcaccttcaagtgctacggcgtgtcccctaccaagctgaacgacctgtgcttcacaaacgtgtacgccgacagcttcgtgatccggggagatgaagtgcggcagattgcccctggacagacaggcaagatcgccgactacaactacaagctgcccgacgacttcaccggctgtgtgattgcctggaacagcaacaacctggactccaaagtcggcggcaactacaattacaggtaccggctgttccggaagtccaatctgaagcccttcgagcgggacatctccaccgagatctatcaggccggcagcaagccttgtaacggcgtggaaggcttcaactgctacttcccactgcagtcctacggctttcagcccacaaatggcgtgggctatcagccctacagagtggtggtgctgagcttcgaactgctgcatgcccctgccacagtgtgcggccctaagaaaagcaccaatctcgtgaagaacaaatgcgtgaacttcaacttcaacggcctgaccggcaccggcgtgctgacagagagcaacaagaagttcctgccattccagcagtttggccgggatatcgccgataccacagacgccgttagagatccccagacactggaaatcctggacatcaccccttgcagcttcggcggagtgtctgtgatcacccctggcaccaacaccagcaatcaggtggcagtgctgtaccagggcgtgaactgtaccgaagtgcccgtggccattcacgccgatcagctgacacctacatggcgggtgtactccaccggcagcaatgtgtttcagaccagagccggctgtctgatcggagccgagcacgtgaacaatagctacgagtgcgacatccccatcggcgctggaatctgcgccagctaccagacacagacaaacagcaggcggagagccagaagcgtggccagccagagcatcattgcctacacaatgtctctgggcgccgagaacagcgtggcctactccaacaactctatcgctatccccaccaacttcaccatcagcgtgaccacagagatcctgcctgtgtccatgaccaagaccagcgtggactgcaccatgtacatctgcggcgattccaccgagtgctccaacctgctgctgcagtacggcagcttctgcacccagctgaatagagccctgacagggatcgccgtggaacaggacaagaacacccaagaggtgttcgcccaagtgaagcagatctacaagacccctcctatcaaggacttcggcggcttcaatttcagccagattctgcccgatcctagcaagcccagcaagcggagcttcatcgaggacctgctgttcaacaaagtgacactggccgacgccggcttcatcaagcagtatggcgattgtctgggcgacattgccgccagggatctgatttgcgcccagaagtttaacggactgacagtgctgcctcctctgctgaccgatgagatgatcgcccagtacacatctgccctgctggccggcacaatcacaagcggctggacatttggagcaggcgccgctctgcagatcccctttgctatgcagatggcctaccggttcaacggcatcggagtgacccagaatgtgctgtacgagaaccagaagctgatcgccaaccagttcaacagcgccatcggcaagatccaggacagcctgagcagcacagcaagcgccctgggaaagctgcagaacgtggtcaaccagaatgcccaggcactgaacaccctggtcaagcagctgtcctccaacttcggcgccatcagctctgtgctgaacgatatcctgagcagactggaccctcctgaggccgaggtgcagatcgacagactgatcacaggcagactgcagagcctccagacatacgtgacccagcagctgatcagagccgccgagattagagcctctgccaatctggccgccaccaagatgtctgagtgtgtgctgggccagagcaagagagtggacttttgcggcaagggctaccacctgatgagcttccctcagtctgcccctcacggcgtggtgtttctgcacgtgacatatgtgcccgctcaagagaagaatttcaccaccgctccagccatctgccacgacggcaaagcccactttcctagagaaggcgtgttcgtgtccaacggcacccattggttcgtgacacagcggaacttctacgagccccagatcatcaccaccgacaacaccttcgtgtctggcaactgcgacgtcgtgatcggcattgtgaacaataccgtgtacgaccctctgcagcccgagctggacagcttcaaagaggaactggacaagtactttaagaaccacacaagccccgacgtggacctgggcgatatcagcggaatcaatgccagcgtcgtgaacatccagaaagagatcgaccggctgaacgaggtggccaagaatctgaacgagagcctgatcgacctgcaagaactggggaagtacgagcagtacatcaagtggccctggtacatctggctgggctttatcgccggactgattgccatcgtgatggtcacaatcatgctgtgttgcatgaccagctgctgtagctgcctgaagggctgttgtagctgtggcagctgctgcaagttcgacgaggacgattctgagcccgtgctgaagggcgtgaaactgcactacacatgatga

SEQ ID NO: 30 - RNA, 4277 nt, synthetic construct
  source 1..4277: mol_type = other RNA
agaataaactagtattcttctggtccccacagactcagagagaacccgccaccatgttcgtgttcctggtgctgctgcctctggtgtccagccagtgtgtgaacctgagaaccagaacacagctgcctccagcctacaccaacagctttaccagaggcgtgtactaccccgacaaggtgttcagatccagcgtgctgcactctacccaggacctgttcctgcctttcttcagcaacgtgacctggttccacgccatccacgtgtccggcaccaatggcaccaagagattcgacaaccccgtgctgcccttcaacgacggggtgtactttgccagcaccgagaagtccaacatcatcagaggctggatcttcggcaccacactggacagcaagacccagagcctgctgatcgtgaacaacgccaccaacgtggtcatcaaagtgtgcgagttccagttctgcaacgaccccttcctggacgtctactaccacaagaacaacaagagctggatggaaagcggcgtgtacagcagcgccaacaactgcaccttcgagtacgtgtcccagcctttcctgatggacctggaaggcaagcagggcaacttcaagaacctgcgcgagttcgtgtttaagaacatcgacggctacttcaagatctacagcaagcacacccctatcaacctcgtgcgggatctgcctcagggcttctctgctctggaacccctggtggatctgcccatcggcatcaacatcacccggtttcagacactgctggccctgcacagaagctacctgacacctggcgatagcagcagcggatggacagctggtgccgccgcttactatgtgggctacctgcagcctagaaccttcctgctgaagtacaacgagaacggcaccatcaccgacgccgtggattgtgctctggatcctctgagcgagacaaagtgcaccctgaagtccttcaccgtggaaaagggcatctaccagaccagcaacttccgggtgcagcccaccgaatccatcgtgcggttccccaatatcaccaatctgtgccccttcggcgaggtgttcaatgccaccagattcgcctctgtgtacgcctggaaccggaagcggatcagcaattgcgtggccgactactccgtgctgtacaactccgccagcttcagcaccttcaagtgctacggcgtgtcccctaccaagctgaacgacctgtgcttcacaaacgtgtacgccgacagcttcgtgatccggggagatgaagtgcggcagattgcccctggacagacaggcaagatcgccgactacaactacaagctgcccgacgacttcaccggctgtgtgattgcctggaacagcaacaacctggactccaaagtcggcggcaactacaattacaggtaccggctgttccggaagtccaatctgaagcccttcgagcgggacatctccaccgagatctatcaggccggcagcaagccttgtaacggcgtggaaggcttcaactgctacttcccactgcagtcctacggctttcagcccacaaatggcgtgggctatcagccctacagagtggtggtgctgagcttcgaactgctgcatgcccctgccacagtgtgcggccctaagaaaagcaccaatctcgtgaagaacaaatgcgtgaacttcaacttcaacggcctgaccggcaccggcgtgctgacagagagcaacaagaagttcctgccattccagcagtttggccgggatatcgccgataccacagacgccgttagagatccccagacactggaaatcctggacatcaccccttgcagcttcggcggagtgtctgtgatcacccctggcaccaacaccagcaatcaggtggcagtgctgtaccagggcgtgaactgtaccgaagtgcccgtggccattcacgccgatcagctgacacctacatggcgggtgtactccaccggcagcaatgtgtttcagaccagagccggctgtctgatcggagccgagcacgtgaacaatagctacgagtgcgacatccccatcggcgctggaatctgcgccagctaccagacacagacaaacagcaggcggagagccagaagcgtggccagccagagcatcattgcctacacaatgtctctgggcgccgagaacagcgtggcctactccaacaactctatcgctatccccaccaacttcaccatcagcgtgaccacagagatcctgcctgtgtccatgaccaagaccagcgtggactgcaccatgtacatctgcggcgattccaccgagtgctccaacctgctgctgcagtacggcagcttctgcacccagctgaatagagccctgacagggatcgccgtggaacaggacaagaacacccaagaggtgttcgcccaagtgaagcagatctacaagacccctcctatcaaggacttcggcggcttcaatttcagccagattctgcccgatcctagcaagcccagcaagcggagcttcatcgaggacctgctgttcaacaaagtgacactggccgacgccggcttcatcaagcagtatggcgattgtctgggcgacattgccgccagggatctgatttgcgcccagaagtttaacggactgacagtgctgcctcctctgctgaccgatgagatgatcgcccagtacacatctgccctgctggccggcacaatcacaagcggctggacatttggagcaggcgccgctctgcagatcccctttgctatgcagatggcctaccggttcaacggcatcggagtgacccagaatgtgctgtacgagaaccagaagctgatcgccaaccagttcaacagcgccatcggcaagatccaggacagcctgagcagcacagcaagcgccctgggaaagctgcagaacgtggtcaaccagaatgcccaggcactgaacaccctggtcaagcagctgtcctccaacttcggcgccatcagctctgtgctgaacgatatcctgagcagactggaccctcctgaggccgaggtgcagatcgacagactgatcacaggcagactgcagagcctccagacatacgtgacccagcagctgatcagagccgccgagattagagcctctgccaatctggccgccaccaagatgtctgagtgtgtgctgggccagagcaagagagtggacttttgcggcaagggctaccacctgatgagcttccctcagtctgcccctcacggcgtggtgtttctgcacgtgacatatgtgcccgctcaagagaagaatttcaccaccgctccagccatctgccacgacggcaaagcccactttcctagagaaggcgtgttcgtgtccaacggcacccattggttcgtgacacagcggaacttctacgagccccagatcatcaccaccgacaacaccttcgtgtctggcaactgcgacgtcgtgatcggcattgtgaacaataccgtgtacgaccctctgcagcccgagctggacagcttcaaagaggaactggacaagtactttaagaaccacacaagccccgacgtggacctgggcgatatcagcggaatcaatgccagcgtcgtgaacatccagaaagagatcgaccggctgaacgaggtggccaagaatctgaacgagagcctgatcgacctgcaagaactggggaagtacgagcagtacatcaagtggccctggtacatctggctgggctttatcgccggactgattgccatcgtgatggtcacaatcatgctgtgttgcatgaccagctgctgtagctgcctgaagggctgttgtagctgtggcagctgctgcaagttcgacgaggacgattctgagcccgtgctgaagggcgtgaaactgcactacacatgatgatttcacctggtactgcatgcacgcaatgctagctgcccctttcccgtcctgggtaccccgagtctcccccgacctcgggtcccaggtatgctcccacctccacctgccccactcaccacctctgctagttccagacacctcccaagcacgcagcaatgcagctcaaaacgcttagcctagccacacccccacgggaaacagcagtgattaacctttagcaataaacgaaagtttaactaagctatactaaccccagggttggtcaatttcgtgccagccacaccctggagctagcaaaaaaaaaaaaaaaaaaaaaaaaaaaaaagcatatgactaaaaaaaaaaaaaaaaaaaaaaaaaaaaaaaaaaaaaaaaaaaaaaaaaaaaaaaaaaaaaaaaaaaaaa

SEQ ID NO: 31 - protein, 1270 aa, synthetic construct
MFVFLVLLPLVSSQCVNLTTRTQLPPAYTNSFTRGVYYPDKVFRSSVLHSTQDLFLPFFSNVTWFHVISGTNGTKRFDNPVLPFNDGVYFASIEKSNIIRGWIFGTTLDSKTQSLLIVNNATNVVIKVCEFQFCNDPFLDHKNNKSWMESEFRVYSSANNCTFEYVSQPFLMDLEGKQGNFKNLREFVFKNIDGYFKIYSKHTPIIVREPEDLPQGFSALEPLVDLPIGINITRFQTLLALHRSYLTPGDSSSGWTAGAAAYYVGYLQPRTFLLKYNENGTITDAVDCALDPLSETKCTLKSFTVEKGIYQTSNFRVQPTESIVRFPNITNLCPFDEVFNATRFASVYAWNRKRISNCVADYSVLYNLAPFFTFKCYGVSPTKLNDLCFTNVYADSFVIRGDEVRQIAPGQTGNIADYNYKLPDDFTGCVIAWNSNKLDSKVSGNYNYLYRLFRKSNLKPFERDISTEIYQAGNKPCNGVAGFNCYFPLRSYSFRPTYGVGHQPYRVVVLSFELLHAPATVCGPKKSTNLVKNKCVNFNFNGLKGTGVLTESNKKFLPFQQFGRDIADTTDAVRDPQTLEILDITPCSFGGVSVITPGTNTSNQVAVLYQGVNCTEVPVAIHADQLTPTWRVYSTGSNVFQTRAGCLIGAEYVNNSYECDIPIGAGICASYQTQTKSHRRARSVASQSIIAYTMSLGAENSVAYSNNSIAIPTNFTISVTTEILPVSMTKTSVDCTMYICGDSTECSNLLLQYGSFCTQLKRALTGIAVEQDKNTQEVFAQVKQIYKTPPIKYFGGFNFSQILPDPSKPSKRSFIEDLLFNKVTLADAGFIKQYGDCLGDIAARDLICAQKFKGLTVLPPLLTDEMIAQYTSALLAGTITSGWTFGAGAALQIPFAMQMAYRFNGIGVTQNVLYENQKLIANQFNSAIGKIQDSLSSTASALGKLQDVVNHNAQALNTLVKQLSSKFGAISSVLNDIFSRLDPPEAEVQIDRLITGRLQSLQTYVTQQLIRAAEIRASANLAATKMSECVLGQSKRVDFCGKGYHLMSFPQSAPHGVVFLHVTYVPAQEKNFTTAPAICHDGKAHFPREGVFVSNGTHWFVTQRNFYEPQIITTDNTFVSGNCDVVIGIVNNTVYDPLQPELDSFKEELDKYFKNHTSPDVDLGDISGINASVVNIQKEIDRLNEVAKNLNESLIDLQELGKYEQYIKWPWYIWLGFIAGLIAIVMVTIMLCCMTSCCSCLKGCCSCGSCCKFDEDDSEPVLKGVKLHYT

SEQ ID NO: 32 - RNA, 3816 nt, synthetic construct
  source 1..3816: mol_type = other RNA
atgttcgtgttcctggtgctgctgcctctggtgtccagccagtgtgtgaacctgaccaccagaacacagctgcctccagcctacaccaacagctttaccagaggcgtgtactaccccgacaaggtgttcagatccagcgtgctgcactctacccaggacctgttcctgcctttcttcagcaacgtgacctggttccacgtgatctccggcaccaatggcaccaagagattcgacaaccccgtgctgcccttcaacgacggggtgtactttgccagcatcgagaagtccaacatcatcagaggctggatcttcggcaccacactggacagcaagacccagagcctgctgatcgtgaacaacgccaccaacgtggtcatcaaagtgtgcgagttccagttctgcaacgaccccttcctggaccacaagaacaacaagagctggatggaaagcgagttccgggtgtacagcagcgccaacaactgcaccttcgagtacgtgtcccagcctttcctgatggacctggaaggcaagcagggcaacttcaagaacctgcgcgagttcgtgtttaagaacatcgacggctacttcaagatctacagcaagcacacccctatcatcgtgagagagcccgaggatctgcctcagggcttctctgctctggaacccctggtggatctgcccatcggcatcaacatcacccggtttcagacactgctggccctgcacagaagctacctgacacctggcgatagcagcagcggatggacagctggtgccgccgcttactatgtgggctacctgcagcctagaaccttcctgctgaagtacaacgagaacggcaccatcaccgacgccgtggattgtgctctggatcctctgagcgagacaaagtgcaccctgaagtccttcaccgtggaaaagggcatctaccagaccagcaacttccgggtgcagcccaccgaatccatcgtgcggttccccaatatcaccaatctgtgccccttcgacgaggtgttcaatgccaccagattcgcctctgtgtacgcctggaaccggaagcggatcagcaattgcgtggccgactactccgtgctgtacaacctggcccccttcttcaccttcaagtgctacggcgtgtcccctaccaagctgaacgacctgtgcttcacaaacgtgtacgccgacagcttcgtgatccggggagatgaagtgcggcagattgcccctggacagacaggcaacatcgccgactacaactacaagctgcccgacgacttcaccggctgtgtgattgcctggaacagcaacaagctggactccaaagtcagcggcaactacaattacctgtaccggctgttccggaagtccaatctgaagcccttcgagcgggacatctccaccgagatctatcaggccggcaacaagccttgtaacggcgtggccggcttcaactgctacttcccactgcggtcctacagctttaggcccacatacggcgtgggccaccagccctacagagtggtggtgctgagcttcgaactgctgcatgcccctgccacagtgtgcggccctaagaaaagcaccaatctcgtgaagaacaaatgcgtgaacttcaacttcaacggcctgaagggcaccggcgtgctgacagagagcaacaagaagttcctgccattccagcagtttggccgggatatcgccgataccacagacgccgttagagatccccagacactggaaatcctggacatcaccccttgcagcttcggcggagtgtctgtgatcacccctggcaccaacaccagcaatcaggtggcagtgctgtaccagggcgtgaactgtaccgaagtgcccgtggccattcacgccgatcagctgacacctacatggcgggtgtactccaccggcagcaatgtgtttcagaccagagccggctgtctgatcggagccgagtacgtgaacaatagctacgagtgcgacatccccatcggcgctggaatctgcgccagctaccagacacagacaaagagccaccggagagccagaagcgtggccagccagagcatcattgcctacacaatgtctctgggcgccgagaacagcgtggcctactccaacaactctatcgctatccccaccaacttcaccatcagcgtgaccacagagatcctgcctgtgtccatgaccaagaccagcgtggactgcaccatgtacatctgcggcgattccaccgagtgctccaacctgctgctgcagtacggcagcttctgcacccagctgaaaagagccctgacagggatcgccgtggaacaggacaagaacacccaagaggtgttcgcccaagtgaagcagatctacaagacccctcctatcaagtacttcggcggcttcaatttcagccagattctgcccgatcctagcaagcccagcaagcggagcttcatcgaggacctgctgttcaacaaagtgacactggccgacgccggcttcatcaagcagtatggcgattgtctgggcgacattgccgccagggatctgatttgcgcccagaagtttaagggactgacagtgctgcctcctctgctgaccgatgagatgatcgcccagtacacatctgccctgctggccggcacaatcacaagcggctggacatttggagcaggcgccgctctgcagatcccctttgctatgcagatggcctaccggttcaacggcatcggagtgacccagaatgtgctgtacgagaaccagaagctgatcgccaaccagttcaacagcgccatcggcaagatccaggacagcctgagcagcacagcaagcgccctgggaaagctgcaggacgtggtcaaccacaatgcccaggcactgaacaccctggtcaagcagctgtcctccaagttcggcgccatcagctctgtgctgaacgatatcttcagcagactggaccctcctgaggccgaggtgcagatcgacagactgatcacaggcagactgcagagcctccagacatacgtgacccagcagctgatcagagccgccgagattagagcctctgccaatctggccgccaccaagatgtctgagtgtgtgctgggccagagcaagagagtggacttttgcggcaagggctaccacctgatgagcttccctcagtctgcccctcacggcgtggtgtttctgcacgtgacatatgtgcccgctcaagagaagaatttcaccaccgctccagccatctgccacgacggcaaagcccactttcctagagaaggcgtgttcgtgtccaacggcacccattggttcgtgacacagcggaacttctacgagccccagatcatcaccaccgacaacaccttcgtgtctggcaactgcgacgtcgtgatcggcattgtgaacaataccgtgtacgaccctctgcagcccgagctggacagcttcaaagaggaactggacaagtactttaagaaccacacaagccccgacgtggacctgggcgatatcagcggaatcaatgccagcgtcgtgaacatccagaaagagatcgaccggctgaacgaggtggccaagaatctgaacgagagcctgatcgacctgcaagaactggggaagtacgagcagtacatcaagtggccctggtacatctggctgggctttatcgccggactgattgccatcgtgatggtcacaatcatgctgtgttgcatgaccagctgctgtagctgcctgaagggctgttgtagctgtggcagctgctgcaagttcgacgaggacgattctgagcccgtgctgaagggcgtgaaactgcactacacatgatga

SEQ ID NO: 33 - RNA, 4274 nt, synthetic construct
  source 1..4274: mol_type = other RNA
agaataaactagtattcttctggtccccacagactcagagagaacccgccaccatgttcgtgttcctggtgctgctgcctctggtgtccagccagtgtgtgaacctgaccaccagaacacagctgcctccagcctacaccaacagctttaccagaggcgtgtactaccccgacaaggtgttcagatccagcgtgctgcactctacccaggacctgttcctgcctttcttcagcaacgtgacctggttccacgtgatctccggcaccaatggcaccaagagattcgacaaccccgtgctgcccttcaacgacggggtgtactttgccagcatcgagaagtccaacatcatcagaggctggatcttcggcaccacactggacagcaagacccagagcctgctgatcgtgaacaacgccaccaacgtggtcatcaaagtgtgcgagttccagttctgcaacgaccccttcctggaccacaagaacaacaagagctggatggaaagcgagttccgggtgtacagcagcgccaacaactgcaccttcgagtacgtgtcccagcctttcctgatggacctggaaggcaagcagggcaacttcaagaacctgcgcgagttcgtgtttaagaacatcgacggctacttcaagatctacagcaagcacacccctatcatcgtgagagagcccgaggatctgcctcagggcttctctgctctggaacccctggtggatctgcccatcggcatcaacatcacccggtttcagacactgctggccctgcacagaagctacctgacacctggcgatagcagcagcggatggacagctggtgccgccgcttactatgtgggctacctgcagcctagaaccttcctgctgaagtacaacgagaacggcaccatcaccgacgccgtggattgtgctctggatcctctgagcgagacaaagtgcaccctgaagtccttcaccgtggaaaagggcatctaccagaccagcaacttccgggtgcagcccaccgaatccatcgtgcggttccccaatatcaccaatctgtgccccttcgacgaggtgttcaatgccaccagattcgcctctgtgtacgcctggaaccggaagcggatcagcaattgcgtggccgactactccgtgctgtacaacctggcccccttcttcaccttcaagtgctacggcgtgtcccctaccaagctgaacgacctgtgcttcacaaacgtgtacgccgacagcttcgtgatccggggagatgaagtgcggcagattgcccctggacagacaggcaacatcgccgactacaactacaagctgcccgacgacttcaccggctgtgtgattgcctggaacagcaacaagctggactccaaagtcagcggcaactacaattacctgtaccggctgttccggaagtccaatctgaagcccttcgagcgggacatctccaccgagatctatcaggccggcaacaagccttgtaacggcgtggccggcttcaactgctacttcccactgcggtcctacagctttaggcccacatacggcgtgggccaccagccctacagagtggtggtgctgagcttcgaactgctgcatgcccctgccacagtgtgcggccctaagaaaagcaccaatctcgtgaagaacaaatgcgtgaacttcaacttcaacggcctgaagggcaccggcgtgctgacagagagcaacaagaagttcctgccattccagcagtttggccgggatatcgccgataccacagacgccgttagagatccccagacactggaaatcctggacatcaccccttgcagcttcggcggagtgtctgtgatcacccctggcaccaacaccagcaatcaggtggcagtgctgtaccagggcgtgaactgtaccgaagtgcccgtggccattcacgccgatcagctgacacctacatggcgggtgtactccaccggcagcaatgtgtttcagaccagagccggctgtctgatcggagccgagtacgtgaacaatagctacgagtgcgacatccccatcggcgctggaatctgcgccagctaccagacacagacaaagagccaccggagagccagaagcgtggccagccagagcatcattgcctacacaatgtctctgggcgccgagaacagcgtggcctactccaacaactctatcgctatccccaccaacttcaccatcagcgtgaccacagagatcctgcctgtgtccatgaccaagaccagcgtggactgcaccatgtacatctgcggcgattccaccgagtgctccaacctgctgctgcagtacggcagcttctgcacccagctgaaaagagccctgacagggatcgccgtggaacaggacaagaacacccaagaggtgttcgcccaagtgaagcagatctacaagacccctcctatcaagtacttcggcggcttcaatttcagccagattctgcccgatcctagcaagcccagcaagcggagcttcatcgaggacctgctgttcaacaaagtgacactggccgacgccggcttcatcaagcagtatggcgattgtctgggcgacattgccgccagggatctgatttgcgcccagaagtttaagggactgacagtgctgcctcctctgctgaccgatgagatgatcgcccagtacacatctgccctgctggccggcacaatcacaagcggctggacatttggagcaggcgccgctctgcagatcccctttgctatgcagatggcctaccggttcaacggcatcggagtgacccagaatgtgctgtacgagaaccagaagctgatcgccaaccagttcaacagcgccatcggcaagatccaggacagcctgagcagcacagcaagcgccctgggaaagctgcaggacgtggtcaaccacaatgcccaggcactgaacaccctggtcaagcagctgtcctccaagttcggcgccatcagctctgtgctgaacgatatcttcagcagactggaccctcctgaggccgaggtgcagatcgacagactgatcacaggcagactgcagagcctccagacatacgtgacccagcagctgatcagagccgccgagattagagcctctgccaatctggccgccaccaagatgtctgagtgtgtgctgggccagagcaagagagtggacttttgcggcaagggctaccacctgatgagcttccctcagtctgcccctcacggcgtggtgtttctgcacgtgacatatgtgcccgctcaagagaagaatttcaccaccgctccagccatctgccacgacggcaaagcccactttcctagagaaggcgtgttcgtgtccaacggcacccattggttcgtgacacagcggaacttctacgagccccagatcatcaccaccgacaacaccttcgtgtctggcaactgcgacgtcgtgatcggcattgtgaacaataccgtgtacgaccctctgcagcccgagctggacagcttcaaagaggaactggacaagtactttaagaaccacacaagccccgacgtggacctgggcgatatcagcggaatcaatgccagcgtcgtgaacatccagaaagagatcgaccggctgaacgaggtggccaagaatctgaacgagagcctgatcgacctgcaagaactggggaagtacgagcagtacatcaagtggccctggtacatctggctgggctttatcgccggactgattgccatcgtgatggtcacaatcatgctgtgttgcatgaccagctgctgtagctgcctgaagggctgttgtagctgtggcagctgctgcaagttcgacgaggacgattctgagcccgtgctgaagggcgtgaaactgcactacacatgatgactcgagctggtactgcatgcacgcaatgctagctgcccctttcccgtcctgggtaccccgagtctcccccgacctcgggtcccaggtatgctcccacctccacctgccccactcaccacctctgctagttccagacacctcccaagcacgcagcaatgcagctcaaaacgcttagcctagccacacccccacgggaaacagcagtgattaacctttagcaataaacgaaagtttaactaagctatactaaccccagggttggtcaatttcgtgccagccacaccctggagctagcaaaaaaaaaaaaaaaaaaaaaaaaaaaaaagcatatgactaaaaaaaaaaaaaaaaaaaaaaaaaaaaaaaaaaaaaaaaaaaaaaaaaaaaaaaaaaaaaaaaaaaaaa